European Patent Application EP 4 321 529 A2, published February 14, 2024. Title: PEPTIDES AND COMBINATION OF PEPTIDES OF NON-CANONICAL ORIGIN FOR USE IN IMMUNOTHERAPY AGAINST DIFFERENT TYPES OF CANCERS. Applicant: immatics biotechnologies GmbH. The sequence listing filed with the application follows.

SEQUENCE LISTING (105 sequences)

SEQ ID NO: 1 - protein, 9 aa, Homo sapiens
KLLDFSTRI

SEQ ID NO: 2 - protein, 9 aa, Homo sapiens
ALLDVLVKL

SEQ ID NO: 3 - protein, 11 aa, Homo sapiens
FLLVPSPIWQL

SEQ ID NO: 4 - protein, 9 aa, Homo sapiens
YLGDSHVLL

SEQ ID NO: 5 - protein, 9 aa, Homo sapiens
LVWEVVESV

SEQ ID NO: 6 - protein, 9 aa, Homo sapiens
ALHDSPVYL

SEQ ID NO: 7 - protein, 11 aa, Homo sapiens
ALWEEVKATSL

SEQ ID NO: 8 - protein, 9 aa, Homo sapiens
ILQSLVPAA

SEQ ID NO: 9 - protein, 10 aa, Homo sapiens
FLQEGDLISV

SEQ ID NO: 10 - protein, 9 aa, Homo sapiens
SLLDKLSGI

SEQ ID NO: 11 - protein, 10 aa, Homo sapiens
ALLPHAPEAV

SEQ ID NO: 12 - protein, 9 aa, Homo sapiens
HLDSMNVSI

SEQ ID NO: 13 - protein, 10 aa, Homo sapiens
FLDEGSLLRL

SEQ ID NO: 14 - protein, 9 aa, Homo sapiens
LLIEVSEEL

SEQ ID NO: 15 - protein, 9 aa, Homo sapiens
NLVMPLLHI

SEQ ID NO: 16 - protein, 12 aa, Homo sapiens
ALLDAEQSPVAL

SEQ ID NO: 17 - protein, 11 aa, Homo sapiens
VLWDLRPSSLI

SEQ ID NO: 18 - protein, 9 aa, Homo sapiens
KMMTFFQGL

SEQ ID NO: 19 - protein, 9 aa, Homo sapiens
MLLPWLPKL

SEQ ID NO: 20 - protein, 9 aa, Homo sapiens
VLISLPGKV

SEQ ID NO: 21 - protein, 9 aa, Homo sapiens
FVFISPSFL

SEQ ID NO: 22 - protein, 9 aa, Homo sapiens
SLYDVPVGA

SEQ ID NO: 23 - protein, 9 aa, Homo sapiens
GLEVLDALL

SEQ ID NO: 24 - protein, 9 aa, Homo sapiens
TLTSLNILL

SEQ ID NO: 25 - protein, 9 aa, Homo sapiens
ISVLNLSAI

SEQ ID NO: 26 - protein, 9 aa, Homo sapiens
KLWTSLVNL

SEQ ID NO: 27 - protein, 10 aa, Homo sapiens
IAAGVPNTDA

SEQ ID NO: 28 - protein, 9 aa, Homo sapiens
SQLEKPETA

SEQ ID NO: 29 - protein, 9 aa, Homo sapiens
LLWEFPSMA

SEQ ID NO: 30 - protein, 9 aa, Homo sapiens
LLRLTLLPL

SEQ ID NO: 31 - protein, 9 aa, Homo sapiens
VVLPIVITL

SEQ ID NO: 32 - protein, 10 aa, Homo sapiens
VLSVSAVLGA

SEQ ID NO: 33 - protein, 9 aa, Homo sapiens
FASERPPSV

SEQ ID NO: 34 - protein, 9 aa, Homo sapiens
LLNVEPAGA

SEQ ID NO: 35 - protein, 9 aa, Homo sapiens
VLLNSNYPV

SEQ ID NO: 36 - protein, 9 aa, Homo sapiens
FQVTRTTGV

SEQ ID NO: 37 - protein, 9 aa, Homo sapiens
KILDEFYNV

SEQ ID NO: 38 - protein, 9 aa, Homo sapiens
SLSAWLPSL

SEQ ID NO: 39 - protein, 9 aa, Homo sapiens
YIYEDEVRL

SEQ ID NO: 40 - protein, 9 aa, Homo sapiens
FTLPFLVNL

SEQ ID NO: 41 - protein, 12 aa, Homo sapiens
LMASEGIWESSL

SEQ ID NO: 42 - protein, 9 aa, Homo sapiens
WITPVIPAL

SEQ ID NO: 43 - protein, 9 aa, Homo sapiens
AIWSTILIA

SEQ ID NO: 44 - protein, 10 aa, Homo sapiens
WLIPRQLAAA

SEQ ID NO: 45 - protein, 9 aa, Homo sapiens
ALYHQSPLL

SEQ ID NO: 46 - protein, 9 aa, Homo sapiens
AMVEIIPKV

SEQ ID NO: 47 - protein, 9 aa, Homo sapiens
ALLPGVPGL

SEQ ID NO: 48 - protein, 9 aa, Homo sapiens
MLAEIHPKA

SEQ ID NO: 49 - protein, 10 aa, Homo sapiens
FLWDPRDVVL

SEQ ID NO: 50 - protein, 9 aa, Homo sapiens
GLASYLDRV

SEQ ID NO: 51 - protein, 9 aa, Homo sapiens
GLLTQVHIL

SEQ ID NO: 52 - protein, 9 aa, Homo sapiens
LAFVSHVLI

SEQ ID NO: 53 - protein, 9 aa, Homo sapiens
TISISLSSV

SEQ ID NO: 54 - protein, 9 aa, Homo sapiens
GLSPDQVFL

SEQ ID NO: 55 - protein, 9 aa, Homo sapiens
MVQQEKLFV

SEQ ID NO: 56 - protein, 9 aa, Homo sapiens
IITNLIVNI

SEQ ID NO: 57 - protein, 9 aa, Homo sapiens
YVLMTSLLL

SEQ ID NO: 58 - protein, 10 aa, Homo sapiens
MIISHRALEL

SEQ ID NO: 59 - protein, 10 aa, Homo sapiens
LAASTTFLGV

SEQ ID NO: 60 - protein, 9 aa, Homo sapiens
LLLATLENL

SEQ ID NO: 61 - protein, 9 aa, Homo sapiens
VLPWQPLLL

SEQ ID NO: 62 - protein, 10 aa, Homo sapiens
SLLGKPGLTI

SEQ ID NO: 63 - protein, 9 aa, Homo sapiens
LSFKRSLSI

SEQ ID NO: 64 - protein, 9 aa, Homo sapiens
LLLALRLSL

SEQ ID NO: 65 - protein, 9 aa, Homo sapiens
IAISQLTFV

SEQ ID NO: 66 - protein, 9 aa, Homo sapiens
ILNELLNSI

SEQ ID NO: 67 - protein, 9 aa, Homo sapiens
ALKELMGPA

SEQ ID NO: 68 - protein, 9 aa, Homo sapiens
KLLADAFKV

SEQ ID NO: 69 - protein, 9 aa, Homo sapiens
LLCPVVLQL

SEQ ID NO: 70 - protein, 9 aa, Homo sapiens
LLLQIEPAA

SEQ ID NO: 71 - protein, 9 aa, Homo sapiens
WLMPVMPAL

SEQ ID NO: 72 - protein, 9 aa, Homo sapiens
YLSFIKILL

SEQ ID NO: 73 - protein, 9 aa, Homo sapiens
STTIINLIL

SEQ ID NO: 74 - protein, 9 aa, Homo sapiens
TLLSYSIPL

SEQ ID NO: 75 - protein, 11 aa, Homo sapiens
TTQEAEKLLER

SEQ ID NO: 76 - protein, 10 aa, Homo sapiens
TEQGPTGVTM

SEQ ID NO: 77 - protein, 11 aa, Homo sapiens
VPAGVDVITEY

SEQ ID NO: 78 - protein, 9 aa, Homo sapiens
GLLPPVRAM

SEQ ID NO: 79 - protein, 9 aa, Homo sapiens
KIQDPGTAF

SEQ ID NO: 80 - protein, 9 aa, Homo sapiens
RDQIVTVSV

SEQ ID NO: 81 - protein, 12 aa, Homo sapiens
SLLGAATVEPPK

SEQ ID NO: 82 - protein, 9 aa, Homo sapiens
LAPQMIIAL

SEQ ID NO: 83 - protein, 8 aa, Homo sapiens
KPRGPTPL

SEQ ID NO: 84 - protein, 10 aa, Homo sapiens
RLCPAAPSEK

SEQ ID NO: 85 - protein, 9 aa, Homo sapiens
VYLLTFPPL

SEQ ID NO: 86 - protein, 8 aa, Homo sapiens
LMIGKRIL

SEQ ID NO: 87 - protein, 12 aa, Homo sapiens
LNLVSETEAMVK

SEQ ID NO: 88 - protein, 10 aa, Homo sapiens
DEQETDAFLL

SEQ ID NO: 89 - protein, 8 aa, Homo sapiens
MIFYVLQK

SEQ ID NO: 90 - protein, 9 aa, Homo sapiens
YLRDFKIKR

SEQ ID NO: 91 - protein, 9 aa, Homo sapiens
SSHFILVTF

SEQ ID NO: 92 - protein, 9 aa, Homo sapiens
ELVAVTSVL

SEQ ID NO: 93 - protein, 8 aa, Homo sapiens
WQKNSMRL

SEQ ID NO: 94 - protein, 8 aa, Homo sapiens
MGRRRNLY

SEQ ID NO: 95 - protein, 8 aa, Homo sapiens
QVKIVTLL

SEQ ID NO: 96 - protein, 10 aa, Homo sapiens
KIIEDLANTV

SEQ ID NO: 97 - protein, 11 aa, Homo sapiens
GLIDDKGTIKL

SEQ ID NO: 98 - protein, 9 aa, Homo sapiens
SLMEVTHDL

SEQ ID NO: 99 - protein, 12 aa, Homo sapiens
ALMDGSESRFFV

SEQ ID NO: 100 - protein, 9 aa, Homo sapiens
SLGPPPVGV

SEQ ID NO: 101 - protein, 10 aa, Homo sapiens
KLPEGHLPEV

SEQ ID NO: 102 - protein, 9 aa, Homo sapiens
GLDPTQFRV

SEQ ID NO: 103 - protein, 9 aa, Homo sapiens
SLVSYLDKV

SEQ ID NO: 104 - protein, 10 aa, Homo sapiens
ELAGIGILTV

SEQ ID NO: 105 - protein, 9 aa, Homo sapiens
YLLPAIVHI